European Patent Application EP 4 386 008 A1, published June 19, 2024. Title: New mutant of recombinant ganoderma lucidum immunoregulatory protein and application thereof. Applicant: Changchun Intellicrown Pharmaceutical Co., Ltd. The sequence listing filed with the application follows.

SEQUENCE LISTING (33 sequences)

SEQ ID NO: 1 - DNA, 40 bp, synthetic construct
  misc_feature 1..40: note = Forward Primer F
  source 1..40: mol_type = other DNA
ccgctcgagaaaagaatgtctgatactgctttgatcttca

SEQ ID NO: 2 - DNA, 27 bp, synthetic construct
  misc_feature 1..27: note = Reverse Primer R
  source 1..27: mol_type = other DNA
gctctagactagttccattgagcgata

SEQ ID NO: 3 - DNA, 27 bp, synthetic construct
  misc_feature 1..27: note = Forward Primer F3
  source 1..27: mol_type = other DNA
ccgctcgagaaaagagaggctgaagct

SEQ ID NO: 4 - DNA, 23 bp, synthetic construct
  misc_feature 1..23: note = Reverse Primer R3
  source 1..23: mol_type = other DNA
gctctagatcactagttccattg

SEQ ID NO: 5 - DNA, 23 bp, synthetic construct
  misc_feature 1..23: note = Forward Primer M13F
  source 1..23: mol_type = other DNA
cccagtcacgacgttgtaaaacg

SEQ ID NO: 6 - DNA, 23 bp, synthetic construct
  misc_feature 1..23: note = Reverse Primer M13R
  source 1..23: mol_type = other DNA
agcggataacaatttcacacagg

SEQ ID NO: 7 - DNA, 70 bp, synthetic construct
  misc_feature 1..70: note = Forward Primer F2
  source 1..70: mol_type = other DNA
ccgctcgagaaaagagaagaggccgaagccgaagcagaacctaaaatgtctgatactgctttgatcttca

SEQ ID NO: 8 - protein, 4 aa, synthetic construct
  REGION 1..4: note = spacer peptide sequence 1
EAEA

SEQ ID NO: 9 - protein, 10 aa, synthetic construct
  REGION 1..10: note = spacer peptide sequence 2
EEAEAEAEPK

SEQ ID NO: 10 - protein, 111 aa, synthetic construct
  REGION 1..111: note = rLZ-8
MSDTALIFRLAWDVKKLSFDYTPNWGRGNPNNFIDTVTFPKVLTDKAYTYRVAVSGRNLGVKPSYAVESDGSQKVNFLEYNSGYGIADTNTIQVFVVDPDTNNDFIIAQWN

SEQ ID NO: 11 - protein, 115 aa, synthetic construct
  REGION 1..115: note = EAEA-rLZ-8
EAEAMSDTALIFRLAWDVKKLSFDYTPNWGRGNPNNFIDTVTFPKVLTDKAYTYRVAVSGRNLGVKPSYAVESDGSQKVNFLEYNSGYGIADTNTIQVFVVDPDTNNDFIIAQWN

SEQ ID NO: 12 - protein, 121 aa, synthetic construct
  REGION 1..121: note = EEAEAEAEPK-rLZ-8
EEAEAEAEPKMSDTALIFRLAWDVKKLSFDYTPNWGRGNPNNFIDTVTFPKVLTDKAYTYRVAVSGRNLGVKPSYAVESDGSQKVNFLEYNSGYGIADTNTIQVFVVDPDTNNDFIIAQWN

SEQ ID NO: 13 - protein, 111 aa, synthetic construct
  REGION 1..111: note = rLZ-8 mutant (D70K)
MSDTALIFRLAWDVKKLSFDYTPNWGRGNPNNFIDTVTFPKVLTDKAYTYRVAVSGRNLGVKPSYAVESKGSQKVNFLEYNSGYGIADTNTIQVFVVDPDTNNDFIIAQWN

SEQ ID NO: 14 - protein, 115 aa, synthetic construct
  REGION 1..115: note = EAEA-rLZ-8 mutant (D70K)
EAEAMSDTALIFRLAWDVKKLSFDYTPNWGRGNPNNFIDTVTFPKVLTDKAYTYRVAVSGRNLGVKPSYAVESKGSQKVNFLEYNSGYGIADTNTIQVFVVDPDTNNDFIIAQWN

SEQ ID NO: 15 - protein, 121 aa, synthetic construct
  REGION 1..121: note = EEAEAEAEPK-rLZ-8 mutant (D70K)
EEAEAEAEPKMSDTALIFRLAWDVKKLSFDYTPNWGRGNPNNFIDTVTFPKVLTDKAYTYRVAVSGRNLGVKPSYAVESKGSQKVNFLEYNSGYGIADTNTIQVFVVDPDTNNDFIIAQWN

SEQ ID NO: 16 - protein, 111 aa, synthetic construct
  REGION 1..111: note = rLZ-8 mutant 1 (R9A)
MSDTALIFALAWDVKKLSFDYTPNWGRGNPNNFIDTVTFPKVLTDKAYTYRVAVSGRNLGVKPSYAVESDGSQKVNFLEYNSGYGIADTNTIQVFVVDPDTNNDFIIAQWN

SEQ ID NO: 17 - protein, 111 aa, synthetic construct
  REGION 1..111: note = rLZ-8 mutant 2 (L17K/D70K)
MSDTALIFRLAWDVKKKSFDYTPNWGRGNPNNFIDTVTFPKVLTDKAYTYRVAVSGRNLGVKPSYAVESKGSQKVNFLEYNSGYGIADTNTIQVFVVDPDTNNDFIIAQWN

SEQ ID NO: 18 - protein, 111 aa, synthetic construct
  REGION 1..111: note = rLZ-8 mutant 3 (D20H)
MSDTALIFRLAWDVKKLSFHYTPNWGRGNPNNFIDTVTFPKVLTDKAYTYRVAVSGRNLGVKPSYAVESDGSQKVNFLEYNSGYGIADTNTIQVFVVDPDTNNDFIIAQWN

SEQ ID NO: 19 - protein, 111 aa, synthetic construct
  REGION 1..111: note = rLZ-8 mutant 4 (L17K)
MSDTALIFRLAWDVKKKSFDYTPNWGRGNPNNFIDTVTFPKVLTDKAYTYRVAVSGRNLGVKPSYAVESDGSQKVNFLEYNSGYGIADTNTIQVFVVDPDTNNDFIIAQWN

SEQ ID NO: 20 - protein, 111 aa, synthetic construct
  REGION 1..111: note = rLZ-8 mutant 5 (K46E/K74E)
MSDTALIFRLAWDVKKLSFDYTPNWGRGNPNNFIDTVTFPKVLTDEAYTYRVAVSGRNLGVKPSYAVESDGSQEVNFLEYNSGYGIADTNTIQVFVVDPDTNNDFIIAQWN

SEQ ID NO: 21 - protein, 111 aa, synthetic construct
  REGION 1..111: note = rLZ-8 mutant 6 (K46E)
MSDTALIFRLAWDVKKLSFDYTPNWGRGNPNNFIDTVTFPKVLTDEAYTYRVAVSGRNLGVKPSYAVESDGSQKVNFLEYNSGYGIADTNTIQVFVVDPDTNNDFIIAQWN

SEQ ID NO: 22 - protein, 115 aa, synthetic construct
  REGION 1..115: note = EAEA+mutant 1 (R9A)
EAEAMSDTALIFALAWDVKKLSFDYTPNWGRGNPNNFIDTVTFPKVLTDKAYTYRVAVSGRNLGVKPSYAVESDGSQKVNFLEYNSGYGIADTNTIQVFVVDPDTNNDFIIAQWN

SEQ ID NO: 23 - protein, 115 aa, synthetic construct
  REGION 1..115: note = EAEA+mutant 2 (L17K/D70K)
EAEAMSDTALIFRLAWDVKKKSFDYTPNWGRGNPNNFIDTVTFPKVLTDKAYTYRVAVSGRNLGVKPSYAVESKGSQKVNFLEYNSGYGIADTNTIQVFVVDPDTNNDFIIAQWN

SEQ ID NO: 24 - protein, 115 aa, synthetic construct
  REGION 1..115: note = EAEA+mutant 3 (D20H)
EAEAMSDTALIFRLAWDVKKLSFHYTPNWGRGNPNNFIDTVTFPKVLTDKAYTYRVAVSGRNLGVKPSYAVESDGSQKVNFLEYNSGYGIADTNTIQVFVVDPDTNNDFIIAQWN

SEQ ID NO: 25 - protein, 115 aa, synthetic construct
  REGION 1..115: note = EAEA+mutant 4 (L17K)
EAEAMSDTALIFRLAWDVKKKSFDYTPNWGRGNPNNFIDTVTFPKVLTDKAYTYRVAVSGRNLGVKPSYAVESDGSQKVNFLEYNSGYGIADTNTIQVFVVDPDTNNDFIIAQWN

SEQ ID NO: 26 - protein, 115 aa, synthetic construct
  REGION 1..115: note = EAEA+mutant 5 (K46E/K74E)
EAEAMSDTALIFRLAWDVKKLSFDYTPNWGRGNPNNFIDTVTFPKVLTDEAYTYRVAVSGRNLGVKPSYAVESDGSQEVNFLEYNSGYGIADTNTIQVFVVDPDTNNDFIIAQWN

SEQ ID NO: 27 - protein, 115 aa, synthetic construct
  REGION 1..115: note = EAEA+mutant 6 (K46E)
EAEAMSDTALIFRLAWDVKKLSFDYTPNWGRGNPNNFIDTVTFPKVLTDEAYTYRVAVSGRNLGVKPSYAVESDGSQKVNFLEYNSGYGIADTNTIQVFVVDPDTNNDFIIAQWN

SEQ ID NO: 28 - protein, 121 aa, synthetic construct
  REGION 1..121: note = EEAEAEAEPK+mutant 1 (R9A)
EEAEAEAEPKMSDTALIFALAWDVKKLSFDYTPNWGRGNPNNFIDTVTFPKVLTDKAYTYRVAVSGRNLGVKPSYAVESDGSQKVNFLEYNSGYGIADTNTIQVFVVDPDTNNDFIIAQWN

SEQ ID NO: 29 - protein, 121 aa, synthetic construct
  REGION 1..121: note = EEAEAEAEPK+mutant 2 (L17K/D70K)
EEAEAEAEPKMSDTALIFRLAWDVKKKSFDYTPNWGRGNPNNFIDTVTFPKVLTDKAYTYRVAVSGRNLGVKPSYAVESKGSQKVNFLEYNSGYGIADTNTIQVFVVDPDTNNDFIIAQWN

SEQ ID NO: 30 - protein, 121 aa, synthetic construct
  REGION 1..121: note = EEAEAEAEPK+mutant 3 (D20H)
EEAEAEAEPKMSDTALIFRLAWDVKKLSFHYTPNWGRGNPNNFIDTVTFPKVLTDKAYTYRVAVSGRNLGVKPSYAVESDGSQKVNFLEYNSGYGIADTNTIQVFVVDPDTNNDFIIAQWN

SEQ ID NO: 31 - protein, 121 aa, synthetic construct
  REGION 1..121: note = EEAEAEAEPK+mutant 4 (L17K)
EEAEAEAEPKMSDTALIFRLAWDVKKKSFDYTPNWGRGNPNNFIDTVTFPKVLTDKAYTYRVAVSGRNLGVKPSYAVESDGSQKVNFLEYNSGYGIADTNTIQVFVVDPDTNNDFIIAQWN

SEQ ID NO: 32 - protein, 121 aa, synthetic construct
  REGION 1..121: note = EEAEAEAEPK+mutant 5 (K46E/K74E)
EEAEAEAEPKMSDTALIFRLAWDVKKLSFDYTPNWGRGNPNNFIDTVTFPKVLTDEAYTYRVAVSGRNLGVKPSYAVESDGSQEVNFLEYNSGYGIADTNTIQVFVVDPDTNNDFIIAQWN

SEQ ID NO: 33 - protein, 121 aa, synthetic construct
  REGION 1..121: note = EEAEAEAEPK+mutant 6 (K46E)
EEAEAEAEPKMSDTALIFRLAWDVKKLSFDYTPNWGRGNPNNFIDTVTFPKVLTDEAYTYRVAVSGRNLGVKPSYAVESDGSQKVNFLEYNSGYGIADTNTIQVFVVDPDTNNDFIIAQWN